European Patent Application EP 4 119 682 A1, published January 18, 2023. Title: A METHOD FOR DETERMINING THE DNA IMPURITIES NATURE INSIDE VIRAL PARTICLES. Applicant: GENETHON. The sequence listing filed with the application follows.

SEQUENCE LISTING (24 sequences)

SEQ ID NO: 1 - DNA, 19 bp, Artificial Sequence
  GFP/VG spé forward primer
agtccgccctgagcaaaga

SEQ ID NO: 2 - DNA, 18 bp, Artificial Sequence
  GFP/VG spé reverse primer
gcggtcacgaactccagc

SEQ ID NO: 3 - DNA, 25 bp, Artificial Sequence
  GFP/VG spé probe
caacgagaagcgcgatcacatggtc

SEQ ID NO: 4 - DNA, 21 bp, Artificial Sequence
  KanaR/Kana forward primer
gggcgcccggttctttttgtc

SEQ ID NO: 5 - DNA, 23 bp, Artificial Sequence
  KanaR/Kana reverse primer
gccagtcccttcccgcttcagtg

SEQ ID NO: 6 - DNA, 20 bp, Artificial Sequence
  KanaR/Kana probe
ccgacctgtccggtgccctg

SEQ ID NO: 7 - DNA, 20 bp, Artificial Sequence
  E1a forward primer
atgccaaaccttgtaccgga

SEQ ID NO: 8 - DNA, 20 bp, Artificial Sequence
  E1a reverse primer
ccctcttcatcctcgtcgtc

SEQ ID NO: 9 - DNA, 26 bp, Artificial Sequence
  E1a probe
atcgatcttacctgccacgaggctgg

SEQ ID NO: 10 - DNA, 20 bp, Artificial Sequence
  ribosomal HEK293 (RIB123) forward primer
gcaattattccccatgaacg

SEQ ID NO: 11 - DNA, 20 bp, Artificial Sequence
  ribosomal HEK293 (RIB123) reverse primer
ggcctcactaaaccatccaa

SEQ ID NO: 12 - DNA, 25 bp, Artificial Sequence
  ribosomal HEK293 (RIB123) probe
aagtccctgccctttgtacacaccg

SEQ ID NO: 13 - DNA, 27 bp, Artificial Sequence
  large T antigen (LTag) forward primer
tttagattggctaagaaacagtgatga

SEQ ID NO: 14 - DNA, 21 bp, Artificial Sequence
  large T antigen (LTag) reverse primer
ttccatgttcttctccccacc

SEQ ID NO: 15 - DNA, 31 bp, Artificial Sequence
  large T antigen (LTag) probe
tgatgaagacagccaggaaaatgctgataaa

SEQ ID NO: 16 - DNA, 26 bp, Artificial Sequence
  phage lambda forward primer
acagcccctcgtttattatttatctc

SEQ ID NO: 17 - DNA, 19 bp, Artificial Sequence
  phage lambda reverse primer
cccggcctttctgttatcc

SEQ ID NO: 18 - DNA, 22 bp, Artificial Sequence
  phage lambda probe
tcagccagccgctgtgctttca

SEQ ID NO: 19 - DNA, 24 bp, Artificial Sequence
  phage M13mp18 forward primer
ccagttcttttgggtattccgtta

SEQ ID NO: 20 - DNA, 25 bp, Artificial Sequence
  M13mp18 reverse primer
gaaaagtaagcagatagccgaacaa

SEQ ID NO: 21 - DNA, 25 bp, Artificial Sequence
  phage M13mp18 probe
gaaaagtaagcagatagccgaacaa

SEQ ID NO: 22 - DNA, 26 bp, Artificial Sequence
  VG3 forward primer
tttgacacttcttacaaacccgtatc

SEQ ID NO: 23 - DNA, 22 bp, Artificial Sequence
  VG3 reverse primer
gaactgtggcaaggaacaggat

SEQ ID NO: 24 - DNA, 19 bp, Artificial Sequence
  VG3 probe
cattgtatactgattctcg